European Patent Specification EP 3 215 521 B1, published October 8, 2025. Title: CD8a AND T CELL RECEPTOR VARIANTS AND METHODS OF USING SAME IN MODULATING IMMUNE CELL RESPONSES. Applicant: DAVILA, Eduardo. The sequence listing filed with the application follows.

SEQUENCE LISTING (24 sequences)

SEQ ID NO: 1 - DNA, 705 bp, Homo sapiens
atggccttaccagtgaccgccttgctcctgccgctggccttgctgctccacgccgccaggccgagccagttccgggtgtcgccgctggatcggacctggaacctgggcgagacagtggagctgaagtgccaggtgctgctgtccaacccgacgtcgggctgctcgtggctcttccagccgcgcggcgccgccgccagtcccaccttcctcctatacctctcccaaaacaagcccaaggcggccgaggggctggacacccagcggttctcgggcaagaggttgggggacaccttcgtcctcaccctgagcgacttccgccgagagaacgagggctactatttctgctcggccctgagcaactccatcatgtacttcagccacttcgtgccggtcttcctgccagcgaagcccaccacgacgccagcgccgcgaccaccaacaccggcgcccaccatcgcgtcgcagcccctgtccctgcgcccagaggcgtgccggccagcggcggggggcgcagtgcacacgagggggctggacttcgcctgtgatatctacatctgggcgcccttggccgggacttgtggggtccttctcctgtcactggttatcaccctttactgcaaccacaggaaccgaagacgtgtttgcaaatgtccccggcctgtggtcaaatcgggagacaagcccagcctttcggcgagatacgtc

SEQ ID NO: 2 - DNA, 609 bp, Artificial Sequence
  Human CD8a without intracellular signaling domain
atggccttaccagtgaccgccttgctcctgccgctggccttgctgctccacgccgccaggccgagccagttccgggtgtcgccgctggatcggacctggaacctgggcgagacagtggagctgaagtgccaggtgctgctgtccaacccgacgtcgggctgctcgtggctcttccagccgcgcggcgccgccgccagtcccaccttcctcctatacctctcccaaaacaagcccaaggcggccgaggggctggacacccagcggttctcgggcaagaggttgggggacaccttcgtcctcaccctgagcgacttccgccgagagaacgagggctactatttctgctcggccctgagcaactccatcatgtacttcagccacttcgtgccggtcttcctgccagcgaagcccaccacgacgccagcgccgcgaccaccaacaccggcgcccaccatcgcgtcgcagcccctgtccctgcgcccagaggcgtgccggccagcggcggggggcgcagtgcacacgagggggctggacttcgcctgtgatatctacatctgggcgcccttggccgggacttgtggggtccttctcctgtcactggttatcacc

SEQ ID NO: 3 - DNA, 1074 bp, Artificial Sequence
  Human CD8a-MyD88 where MyD88 lacks the TIR domain
atggccttaccagtgaccgccttgctcctgccgctggccttgctgctccacgccgccaggccgagccagttccgggtgtcgccgctggatcggacctggaacctgggcgagacagtggagctgaagtgccaggtgctgctgtccaacccgacgtcgggctgctcgtggctcttccagccgcgcggcgccgccgccagtcccaccttcctcctatacctctcccaaaacaagcccaaggcggccgaggggctggacacccagcggttctcgggcaagaggttgggggacaccttcgtcctcaccctgagcgacttccgccgagagaacgagggctactatttctgctcggccctgagcaactccatcatgtacttcagccacttcgtgccggtcttcctgccagcgaagcccaccacgacgccagcgccgcgaccaccaacaccggcgcccaccatcgcgtcgcagcccctgtccctgcgcccagaggcgtgccggccagcggcggggggcgcagtgcacacgagggggctggacttcgcctgtgatatctacatctgggcgcccttggccgggacttgtggggtccttctcctgtcactggttatcaccatggctgcaggaggtcccggcgcggggtctgcggccccggtctcctccacatcctcccttcccctggctgctctcaacatgcgagtgcggcgccgcctgtctctgttcttgaacgtgcggacacaggtggcggccgactggaccgcgctggcggaggagatggactttgagtacttggagatccggcaactggagacacaagcggaccccactggcaggctgctggacgcctggcagggacgccctggcgcctctgtaggccgactgctcgagctgcttaccaagctgggccgcgacgacgtgctgctggagctgggacccagcattgaggaggattgccaaaagtatatcttgaagcagcagcaggaggaggctgagaagcctttacaggtggccgctgtagacagcagtgtcccacggacagcagagctggcgggcatcaccacacttgatgaccccctgggg

SEQ ID NO: 4 - DNA, 744 bp, Mus musculus
atggcctcaccgttgacccgctttctgtcgctgaacctgctgctgctgggtgagtcgattatcctggggagtggagaagctaagccacaggcacccgaactccgaatctttccaaagaaaatggacgccgaacttggtcagaaggtggacctggtatgtgaagtgttggggtccgtttcgcaaggatgctcttggctcttccagaactccagctccaaactcccccagcccaccttcgttgtctatatggcttcatcccacaacaagataacgtgggacgagaagctgaattcgtcgaaactgttttctgccatgagggacacgaataataagtacgttctcaccctgaacaagttcagcaaggaaaacgaaggctactatttctgctcagtcatcagcaactcggtgatgtacttcagttctgtcgtgccagtccttcagaaagtgaactctactactaccaagccagtgctgcgaactccctcacctgtgcaccctaccgggacatctcagccccagagaccagaagattgtcggccccgtggctcagtgaaggggaccggattggacttcgcctgtgatatttacatctgggcacccttggccggaatctgcgtggcccttctgctgtccttgatcatcactctcatctgctaccacaggagccgaaagcgtgtttgcaaatgtcccaggccgctagtcagacaggaaggcaagcccagaccttcagagaaaattgtgtaa

SEQ ID NO: 5 - DNA, 651 bp, Artificial Sequence
  Mouse CD8a without the intracellular signaling domain
atggcctcaccgttgacccgctttctgtcgctgaacctgctgctgctgggtgagtcgattatcctggggagtggagaagctaagccacaggcacccgaactccgaatctttccaaagaaaatggacgccgaacttggtcagaaggtggacctggtatgtgaagtgttggggtccgtttcgcaaggatgctcttggctcttccagaactccagctccaaactcccccagcccaccttcgttgtctatatggcttcatcccacaacaagataacgtgggacgagaagctgaattcgtcgaaactgttttctgccatgagggacacgaataataagtacgttctcaccctgaacaagttcagcaaggaaaacgaaggctactatttctgctcagtcatcagcaactcggtgatgtacttcagttctgtcgtgccagtccttcagaaagtgaactctactactaccaagccagtgctgcgaactccctcacctgtgcaccctaccgggacatctcagccccagagaccagaagattgtcggccccgtggctcagtgaaggggaccggattggacttcgcctgtgatatttacatctgggcacccttggccggaatctgcgtggcccttctgctgtccttgatcatcactctcatc

SEQ ID NO: 6 - DNA, 1116 bp, Artificial Sequence
  Mouse CD8a-human MyD88 where MyD88 lacks TIR domain
atggcctcaccgttgacccgctttctgtcgctgaacctgctgctgctgggtgagtcgattatcctggggagtggagaagctaagccacaggcacccgaactccgaatctttccaaagaaaatggacgccgaacttggtcagaaggtggacctggtatgtgaagtgttggggtccgtttcgcaaggatgctcttggctcttccagaactccagctccaaactcccccagcccaccttcgttgtctatatggcttcatcccacaacaagataacgtgggacgagaagctgaattcgtcgaaactgttttctgccatgagggacacgaataataagtacgttctcaccctgaacaagttcagcaaggaaaacgaaggctactatttctgctcagtcatcagcaactcggtgatgtacttcagttctgtcgtgccagtccttcagaaagtgaactctactactaccaagccagtgctgcgaactccctcacctgtgcaccctaccgggacatctcagccccagagaccagaagattgtcggccccgtggctcagtgaaggggaccggattggacttcgcctgtgatatttacatctgggcacccttggccggaatctgcgtggcccttctgctgtccttgatcatcactctcatcatggctgcaggaggtcccggcgcggggtctgcggccccggtctcctccacatcctcccttcccctggctgctctcaacatgcgagtgcggcgccgcctgtctctgttcttgaacgtgcggacacaggtggcggccgactggaccgcgctggcggaggagatggactttgagtacttggagatccggcaactggagacacaagcggaccccactggcaggctgctggacgcctggcagggacgccctggcgcctctgtaggccgactgctcgagctgcttaccaagctgggccgcgacgacgtgctgctggagctgggacccagcattgaggaggattgccaaaagtatatcttgaagcagcagcaggaggaggctgagaagcctttacaggtggccgctgtagacagcagtgtcccacggacagcagagctggcgggcatcaccacacttgatgaccccctgggg

SEQ ID NO: 7 - DNA, 715 bp, Artificial Sequence
  Human CD8a TM-MyD88
attcgtgccggtcttcctgccagcgaagcccaccacgacgccagcgccgcgaccaccaacaccggcgcccaccatcgcgtcgcagcccctgtccctgcgcccagaggcgtgccggccagcggcggggggcgcagtgcacacgagggggctggacttcgcctgtgatatctacatctgggcgcccttggccgggacttgtggggtccttctcctgtcactggttatcaccctttactgcaaccacaggaacatggctgcaggaggtcccggcgcggggtctgcggccccggtctcctccacatcctcccttcccctggctgctctcaacatgcgagtgcggcgccgcctgtctctgttcttgaacgtgcggacacaggtggcggccgactggaccgcgctggcggaggagatggactttgagtacttggagatccggcaactggagacacaagcggaccccactggcaggctgctggacgcctggcagggacgccctggcgcctctgtaggccgactgctcgagctgcttaccaagctgggccgcgacgacgtgctgctggagctgggacccagcattgaggaggattgccaaaagtatatcttgaagcagcagcaggaggaggctgagaagcctttacaggtggccgctgtagacagcagtgtcccacggacagcagagctggcgggcatcaccacacttgatgaccccctgggg

SEQ ID NO: 8 - DNA, 1254 bp, Artificial Sequence
  Mouse CD8a-human CD28-human 41BB-human CD3zeta
atggcctcaccgttgacccgctttctgtcgctgaacctgctgctgctgggtgagtcgattatcctggggagtggagaagctaagccacaggcacccgaactccgaatctttccaaagaaaatggacgccgaacttggtcagaaggtggacctggtatgtgaagtgttggggtccgtttcgcaaggatgctcttggctcttccagaactccagctccaaactcccccagcccaccttcgttgtctatatggcttcatcccacaacaagataacgtgggacgagaagctgaattcgtcgaaactgttttctgccatgagggacacgaataataagtacgttctcaccctgaacaagttcagcaaggaaaacgaaggctactatttctgctcagtcatcagcaactcggtgatgtacttcagttctgtcgtgccagtccttcagaaagtgaactctactactaccaagccagtgctgcgaactccctcacctgtgcaccctaccgggacatctcagccccagagaccagaagattgtcggccccgtggctcagtgaaggggaccggattggacttcgcctgtgatatttacatctgggcacccttggccggaatctgcgtggcccttctgctgtccttgatcatcactctcatcaggagtaagaggagcaggctcctgcacagtgactacatgaacatgactccccgccgccccgggcccacccgcaagcattaccagccctatgccccaccacgcgacttcgcagcctatcgctcccgtttctctgttgttaaacggggcagaaagaagctcctgtatatattcaaacaaccatttatgagaccagtacaaactactcaagaggaagatggctgtagctgccgatttccagaagaagaagaaggaggatgtgaactgagagtgaagttcagcaggagcgcagacgcccccgcgtaccagcagggccagaaccagctctataacgagctcaatctaggacgaagagaggagtacgatgttttggacaagagacgtggccgggaccctgagatggggggaaagccgagaaggaagaaccctcaggaaggcctgtacaatgaactgcagaaagataagatggcggaggcctacagtgagattgggatgaaaggcgagcgccggaggggcaaggggcacgatggcctttaccagggtctcagtacagccaccaaggacacctacgacgcccttcacatgcaggccctgccccctcgctaa

SEQ ID NO: 9 - DNA, 1722 bp, Artificial Sequence
  Human CD4-MyD88 where MyD88 lacks the TIR domain
atgaaccggggagtcccttttaggcacttgcttctggtgctgcaactggcgctcctcccagcagccactcagggaaagaaagtggtgctgggcaaaaaaggggatacagtggaactgacctgtacagcttcccagaagaagagcatacaattccactggaaaaactccaaccagataaagattctgggaaatcagggctccttcttaactaaaggtccatccaagctgaatgatcgcgctgactcaagaagaagcctttgggaccaaggaaactttcccctgatcatcaagaatcttaagatagaagactcagatacttacatctgtgaagtggaggaccagaaggaggaggtgcaattgctagtgttcggattgactgccaactctgacacccacctgcttcaggggcagagcctgaccctgaccttggagagcccccctggtagtagcccctcagtgcaatgtaggagtccaaggggtaaaaacatacagggggggaagaccctctccgtgtctcagctggagctccaggatagtggcacctggacatgcactgtcttgcagaaccagaagaaggtggagttcaaaatagacatcgtggtgctagctttccagaaggcctccagcatagtctataagaaagagggggaacaggtggagttctccttcccactcgcctttacagttgaaaagctgacgggcagtggcgagctgtggtggcaggcggagagggcttcctcctccaagtcttggatcacctttgacctgaagaacaaggaagtgtctgtaaaacgggttacccaggaccctaagctccagatgggcaagaagctcccgctccacctcaccctgccccaggccttgcctcagtatgctggctctggaaacctcaccctggcccttgaagcgaaaacaggaaagttgcatcaggaagtgaacctggtggtgatgagagccactcagctccagaaaaatttgacctgtgaggtgtggggacccacctcccctaagctgatgctgagtttgaaactggagaacaaggaggcaaaggtctcgaagcgggagaaggcggtgtgggtgctgaaccctgaggcggggatgtggcagtgtctgctgagtgactcgggacaggtcctgctggaatccaacatcaaggttctgcccacatggtccaccccggtgcagccaatggccctgattgtgctggggggcgtcgccggcctcctgcttttcattgggctaggcatcttcttcatggctgcaggaggtcccggcgcggggtctgcggccccggtctcctccacatcctcccttcccctggctgctctcaacatgcgagtgcggcgccgcctgtctctgttcttgaacgtgcggacacaggtggcggccgactggaccgcgctggcggaggagatggactttgagtacttggagatccggcaactggagacacaagcggaccccactggcaggctgctggacgcctggcagggacgccctggcgcctctgtaggccgactgctcgagctgcttaccaagctgggccgcgacgacgtgctgctggagctgggacccagcattgaggaggattgccaaaagtatatcttgaagcagcagcaggaggaggctgagaagcctttacaggtggccgctgtagacagcagtgtcccacggacagcagagctggcgggcatcaccacacttgatgaccccctggggtga

SEQ ID NO: 10 - DNA, 1719 bp, Artificial Sequence
  Mouse CD4-human MyD88 where MyD88 lacks the TIR domain
atgtgccgagccatctctcttaggcgcttgctgctgctgctgctgcagctgtcacaactcctagctgtcactcaagggaagacgctggtgctggggaaggaaggggaatcagcagaactgccctgcgagagttcccagaagaagatcacagtcttcacctggaagttctctgaccagaggaagattctggggcagcatggcaaaggtgtattaattagaggaggttcgccttcgcagtttgatcgttttgattccaaaaaaggggcatgggagaaaggatcgtttcctctcatcatcaataaacttaagatggaagactctcagacttatatctgtgagctggagaacaggaaagaggaggtggagttgtgggtgttcaaagtgaccttcagtccgggtaccagcctgttgcaagggcagagcctgaccctgaccttggatagcaactctaaggtctctaaccccttgacagagtgcaaacacaaaaagggtaaagttgtcagtggttccaaagttctctccatgtccaacctaagggttcaggacagcgacttctggaactgcaccgtgaccctggaccagaaaaagaactggttcggcatgacactctcagtgctgggttttcagagcacagctatcacggcctataagagtgagggagagtcagcggagttctccttcccactcaactttgcagaggaaaacgggtggggagagctgatgtggaaggcagagaaggattctttcttccagccctggatctccttctccataaagaacaaagaggtgtccgtacaaaagtccaccaaagacctcaagctccagctgaaggaaacgctcccactcaccctcaagataccccaggtctcgcttcagtttgctggttctggcaacctgactctgactctggacaaagggacactgcatcaggaagtgaacctggtggtgatgaaagtggctcagctcaacaatactttgacctgtgaggtgatgggacctacctctcccaagatgagactgaccctgaagcaggagaaccaggaggccagggtctctgaggagcagaaagtagttcaagtggtggcccctgagacagggctgtggcagtgtctactgagtgaaggtgataaggtcaagatggactccaggatccaggttttatccagaggggtgaaccagacagtgttcctggcttgcgtgctgggtggctccttcggctttctgggtttccttgggctctgcatcctctgcatggctgcaggaggtcccggcgcggggtctgcggccccggtctcctccacatcctcccttcccctggctgctctcaacatgcgagtgcggcgccgcctgtctctgttcttgaacgtgcggacacaggtggcggccgactggaccgcgctggcggaggagatggactttgagtacttggagatccggcaactggagacacaagcggaccccactggcaggctgctggacgcctggcagggacgccctggcgcctctgtaggccgactgctcgagctgcttaccaagctgggccgcgacgacgtgctgctggagctgggacccagcattgaggaggattgccaaaagtatatcttgaagcagcagcaggaggaggctgagaagcctttacaggtggccgctgtagacagcagtgtcccacggacagcagagctggcgggcatcaccacacttgatgaccccctggggtga

SEQ ID NO: 11 - DNA, 2285 bp, Artificial Sequence
  Human DMF5 TCR-MyD88 where MyD88 lacks the TIR domain
ccgccatgatgaaatccttgagagttttactagtgatcctgtggcttcagttgagctgggtttggagccaacagaaggaggtggagcagaattctggacccctcagtgttccagagggagccattgcctctctcaactgcacttacagtgaccgaggttcccagtccttcttctggtacagacaatattctgggaaaagccctgagttgataatgttcatatactccaatggtgacaaagaagatggaaggtttacagcacagctcaataaagccagccagtatgtttctctgctcatcagagactcccagcccagtgattcagccacctacctctgtgccgtgaacttcggaggaggaaagcttatcttcggacagggaacggagttatctgtgaaacccaatatccagaaccctgaccctgccgtgtaccagctgagagactctaaatccagtgacaagtctgtctgcctattcaccgattttgattctcaaacaaatgtgtcacaaagtaaggattctgatgtgtatatcacagacaaaactgtgctagacatgaggtctatggacttcaagagcaacagtgctgtggcctggagcaacaaatctgactttgcatgtgcaaacgccttcaacaacagcattattccagaagacaccttcttccccagcccagaaagttcctgtgatgtcaagctggtcgagaaaagctttgaaacagatacgaacctaaactttcaaaacctgtcagtgattgggttccgaatcctcctcctgaaggtggccgggtttaatctgctcatgacgctgcggctgtggtccagcagagccaaaagagagggcagaggaagtcttctaacatgcggtgacgtggaggagaatcccggccctatgagaatcaggctcctgtgctgtgtggccttttctctcctgtgggcaggtccagtgattgctgggatcacccaggcaccaacatctcagatcctggcagcaggacggcgcatgacactgagatgtacccaggatatgagacataatgccatgtactggtatagacaagatctaggactggggctaaggctcatccattattcaaatactgcaggtaccactggcaaaggagaagtccctgatggttatagtgtctccagagcaaacacagatgatttccccctcacgttggcgtctgctgtaccctctcagacatctgtgtacttctgtgccagcagcctaagtttcggcactgaagctttctttggacaaggcaccagactcacagttgtagaggacctgaacaaggtgttcccacccgaggtcgctgtgtttgagccatcagaagcagagatctcccacacccaaaaggccacactggtgtgcctggccacaggcttcttccctgaccacgtggagctgagctggtgggtgaatgggaaggaggtgcacagtggggtcagcacggacccgcagcccctcaaggagcagcccgccctcaatgactccagatactgcctgagcagccgcctgagggtctcggccaccttctggcagaacccccgcaaccacttccgctgtcaagtccagttctacgggctctcggagaatgacgagtggacccaggatagggccaaacccgtcacccagatcgtcagcgccgaggcctggggtagagcagactgtggctttacctcggtgtcctaccagcaaggggtcctgtctgccaccatcctctatgagatcctgctagggaaggccaccctgtatgctgtgctggtcagcgcccttgtgttgatggccatggtcaagagaaaggatttcggatccatggctgcaggaggtcccggcgcggggtctgcggccccggtctcctccacatcctcccttcccctggctgctctcaacatgcgagtgcggcgccgcctgtctctgttcttgaacgtgcggacacaggtggcggccgactggaccgcgctggcggaggagatggactttgagtacttggagatccggcaactggagacacaagcggaccccactggcaggctgctggacgcctggcagggacgccctggcgcctctgtaggccgactgctcgagctgcttaccaagctgggccgcgacgacgtgctgctggagctgggacccagcattgaggaggattgccaaaagtatatcttgaagcagcagcaggaggaggctgagaagcctttacaggtggccgctgtagacagcagtgtcccacggacagcagagctggcgggcatcaccacacttgatgaccccctgggg

SEQ ID NO: 12 - protein, 235 aa, Homo sapiens
MALPVTALLLPLALLLHAARPSQFRVSPLDRTWNLGETVELKCQVLLSNPTSGCSWLFQPRGAAASPTFLLYLSQNKPKAAEGLDTQRFSGKRLGDTFVLTLSDFRRENEGYYFCSALSNSIMYFSHFVPVFLPAKPTTTPAPRPPTPAPTIASQPLSLRPEACRPAAGGAVHTRGLDFACDIYIWAPLAGTCGVLLLSLVITLYCNHRNRRRVCKCPRPVVKSGDKPSLSARYV

SEQ ID NO: 13 - protein, 203 aa, Artificial Sequence
  Human CD8a without the intracellular signaling domain
MALPVTALLLPLALLLHAARPSQFRVSPLDRTWNLGETVELKCQVLLSNPTSGCSWLFQPRGAAASPTFLLYLSQNKPKAAEGLDTQRFSGKRLGDTFVLTLSDFRRENEGYYFCSALSNSIMYFSHFVPVFLPAKPTTTPAPRPPTPAPTIASQPLSLRPEACRPAAGGAVHTRGLDFACDIYIWAPLAGTCGVLLLSLVIT

SEQ ID NO: 14 - protein, 358 aa, Artificial Sequence
  Human CD8a-MyD88 where MyD88 lacks the TIR domain
MALPVTALLLPLALLLHAARPSQFRVSPLDRTWNLGETVELKCQVLLSNPTSGCSWLFQPRGAAASPTFLLYLSQNKPKAAEGLDTQRFSGKRLGDTFVLTLSDFRRENEGYYFCSALSNSIMYFSHFVPVFLPAKPTTTPAPRPPTPAPTIASQPLSLRPEACRPAAGGAVHTRGLDFACDIYIWAPLAGTCGVLLLSLVITMAAGGPGAGSAAPVSSTSSLPLAALNMRVRRRLSLFLNVRTQVAADWTALAEEMDFEYLEIRQLETQADPTGRLLDAWQGRPGASVGRLLELLTKLGRDDVLLELGPSIEEDCQKYILKQQQEEAEKPLQVAAVDSSVPRTAELAGITTLDDPLG

SEQ ID NO: 15 - protein, 247 aa, Mus musculus
MASPLTRFLSLNLLLLGESIILGSGEAKPQAPELRIFPKKMDAELGQKVDLVCEVLGSVSQGCSWLFQNSSSKLPQPTFVVYMASSHNKITWDEKLNSSKLFSAMRDTNNKYVLTLNKFSKENEGYYFCSVISNSVMYFSSVVPVLQKVNSTTTKPVLRTPSPVHPTGTSQPQRPEDCRPRGSVKGTGLDFACDIYIWAPLAGICVALLLSLIITLICYHRSRKRVCKCPRPLVRQEGKPRPSEKIV

SEQ ID NO: 16 - protein, 217 aa, Artificial Sequence
  Mouse CD8a without the intracellular signaling domain
MASPLTRFLSLNLLLLGESIILGSGEAKPQAPELRIFPKKMDAELGQKVDLVCEVLGSVSQGCSWLFQNSSSKLPQPTFVVYMASSHNKITWDEKLNSSKLFSAMRDTNNKYVLTLNKFSKENEGYYFCSVISNSVMYFSSVVPVLQKVNSTTTKPVLRTPSPVHPTGTSQPQRPEDCRPRGSVKGTGLDFACDIYIWAPLAGICVALLLSLIITLI

SEQ ID NO: 17 - protein, 372 aa, Artificial Sequence
  Mouse CD8a-human MyD88 where MyD88 lacks TIR domain
MASPLTRFLSLNLLLLGESIILGSGEAKPQAPELRIFPKKMDAELGQKVDLVCEVLGSVSQGCSWLFQNSSSKLPQPTFVVYMASSHNKITWDEKLNSSKLFSAMRDTNNKYVLTLNKFSKENEGYYFCSVISNSVMYFSSVVPVLQKVNSTTTKPVLRTPSPVHPTGTSQPQRPEDCRPRGSVKGTGLDFACDIYIWAPLAGICVALLLSLIITLIMAAGGPGAGSAAPVSSTSSLPLAALNMRVRRRLSLFLNVRTQVAADWTALAEEMDFEYLEIRQLETQADPTGRLLDAWQGRPGASVGRLLELLTKLGRDDVLLELGPSIEEDCQKYILKQQQEEAEKPLQVAAVDSSVPRTAELAGITTLDDPLG

SEQ ID NO: 18 - protein, 238 aa, Artificial Sequence
  Human CD8a TM-MyD88
FVPVFLPAKPTTTPAPRPPTPAPTIASQPLSLRPEACRPAAGGAVHTRGLDFACDIYIWAPLAGTCGVLLLSLVITLYCNHRNMAAGGPGAGSAAPVSSTSSLPLAALNMRVRRRLSLFLNVRTQVAADWTALAEEMDFEYLEIRQLETQADPTGRLLDAWQGRPGASVGRLLELLTKLGRDDVLLELGPSIEEDCQKYILKQQQEEAEKPLQVAAVDSSVPRTAELAGITTLDDPLG

SEQ ID NO: 19 - protein, 417 aa, Artificial Sequence
  Mouse CD8a-human CD28-human 41BB-human CD3zeta
MASPLTRFLSLNLLLLGESIILGSGEAKPQAPELRIFPKKMDAELGQKVDLVCEVLGSVSQGCSWLFQNSSSKLPQPTFVVYMASSHNKITWDEKLNSSKLFSAMRDTNNKYVLTLNKFSKENEGYYFCSVISNSVMYFSSVVPVLQKVNSTTTKPVLRTPSPVHPTGTSQPQRPEDCRPRGSVKGTGLDFACDIYIWAPLAGICVALLLSLIITLIRSKRSRLLHSDYMNMTPRRPGPTRKHYQPYAPPRDFAAYRSRFSVVKRGRKKLLYIFKQPFMRPVQTTQEEDGCSCRFPEEEEGGCELRVKFSRSADAPAYQQGQNQLYNELNLGRREEYDVLDKRRGRDPEMGGKPRRKNPQEGLYNELQKDKMAEAYSEIGMKGERRRGKGHDGLYQGLSTATKDTYDALHMQALPPR

SEQ ID NO: 20 - protein, 575 aa, Artificial Sequence
  Human CD4-MyD88 where MyD88 lacks the TIR domain
METNRGVPFRHLLLVLQLALLPAATQGKKVVLGKKGDTVELTCTASQKKSIQFHWKNSNQIKILGNQGSFLTKGPSKLNDRADSRRSLWDQGNFPLIIKNLKIEDSDTYICEVEDQKEEVQLLVFGLTANSDTHLLQGQSLTLTLESPPGSSPSVQCRSPRGKNIQGGKTLSVSQLELQDSGTWTCTVLQNQKKVEFKIDIVVLAFQKASSIVYKKEGEQVEFSFPLAFTVEKLTGSGELWWQAERASSSKSWITFDLKNKEVSVKRVTQDPKLQMGKKLPLHLTLPQALPQYAGSGNLTLALEAKTGKLHQEVNLVVMRATQLQKNLTCEVWGPTSPKLMLSLKLENKEAKVSKREKAVWVLNPEAGMWQCLLSDSGQVLLESNIKVLPTWSTPVQPMALIVLGGVAGLLLFIGLGIFFMAAGGPGAGSAAPVSSTSSLPLAALNMRVRRRLSLFLNVRTQVAADWTALAEEMDFEYLEIRQLETQADPTGRLLDAWQGRPGASVGRLLELLTKLGRDDVLLELGPSIEEDCQKYILKQQQEEAEKPLQVAAVDSSVPRTAELAGITTLDDPLG

SEQ ID NO: 21 - protein, 576 aa, Artificial Sequence
  Mouse CD4-human MyD88 where MyD88 lacks the TIR domain
METCRAISLRRLLLLLLQLSQLLAVTQGKTLVLGKEGESAELPCESSQKKITVFTWKFSDQRKILGQHGKGVLIRGGSPSQFDRFDSKKGAWEKGSFPLIINKLKMETEDSQTYICELENRKEEVELWVFKVTFSPGTSLLQGQSLTLTLDSNSKVSNPLTECKHKKGKVVSGSKVLSMSNLRVQDSDFWNCTVTLDQKKNWFGMTLSVLGFQSTAITAYKSEGESAEFSFPLNFAEENGWGELMWKAEKDSFFQPWISFSIKNKEVSVQKSTKDLKLQLKETLPLTLKIPQVSLQFAGSGNLTLTLDKGTLHQEVNLVVMKVAQLNNTLTCEVMGPTSPKMRLTLKQENQEARVSEEQKVVQVVAPETGLWQCLLSEGDKVKMDSRIQVLSRGVNQTVFLACVLGGSFGFLGFLGLCILCMAAGGPGAGSAAPVSSTSSLPLAALNMRVRRRLSLFLNVRTQVAADWTALAEEMDFEYLEIRQLETQADPTGRLLDAWQGRPGASVGRLLELLTKLGRDDVLLELGPSIEEDCQKYILKQQQEEAEKPLQVAAVDSSVPRTAELAGITTLDDPLG

SEQ ID NO: 22 - protein, 780 aa, Artificial Sequence
  Human DMF5 TCR-MyD88 where MyD88 lacks the TIR domain
METMETKSLRVLLVILWLQLSWVWSQQKEVEQNSGPLSVPEGAIASLNCTYSDRGSQSFFWYRQYSGKSPELIMETFIYSNGDKEDGRFTAQLNKASQYVSLLIRDSQPSDSATYLCAVNFGGGKLIFGQGTELSVKPNIQNPDPAVYQLRDSKSSDKSVCLFTDFDSQTNVSQSKDSDVYITDKTVLDMETRSMETDFKSNSAVAWSNKSDFACANAFNNSIIPEDTFFPSPESSCDVKLVEKSFETDTNLNFQNLSVIGFRILLLKVAGFNLLMETTLRLWSSRAKREGRGSLLTCGDVEENPGPMETRIRLLCCVAFSLLWAGPVIAGITQAPTSQILAAGRRMETTLRCTQDMETRHNAMYWYRQDLGLGLRLIHYSNTAGTTGKGEVPDGYSVSRANTDDFPLTLASAVPSQTSVYFCASSLSFGTEAFFGQGTRLTVVEDLNKVFPPEVAVFEPSEAEISHTQKATLVCLATGFFPDHVELSWWVNGKEVHSGVSTDPQPLKEQPALNDSRYCLSSRLRVSATFWQNPRNHFRCQVQFYGLSENDEWTQDRAKPVTQIVSAEAWGRADCGFTSVSYQQGVLSATILYEILLGKATLYAVLVSALVLMAMVKRKDFGSMAAGGPGAGSAAPVSSTSSLPLAALNMRVRRRLSLFLNVRTQVAADWTALAEEMDFEYLEIRQLETQADPTGRLLDAWQGRPGASVGRLLELLTKLGRDDVLLELGPSIEEDCQKYILKQQQEEAEKPLQVAAVDSSVPRTAELAGITTLDDPLGGS

SEQ ID NO: 23 - protein, 247 aa, Artificial Sequence
  Mouse CD8a protein with K73A mutation
MASPLTRFLSLNLLLLGESIILGSGEAKPQAPELRIFPKKMDAELGQKVDLVCEVLGSVSQGCSWLFQNSSSALPQPTFVVYMASSHNKITWDEKLNSSKLFSAMRDTNNKYVLTLNKFSKENEGYYFCSVISNSVMYFSSVVPVLQKVNSTTTKPVLRTPSPVHPTGTSQPQRPEDCRPRGSVKGTGLDFACDIYIWAPLAGICVALLLSLIITLICYHRSRKRVCKCPRPLVRQEGKPRPSEKIV

SEQ ID NO: 24 - protein, 296 aa, Homo sapiens
MAAGGPGAGSAAPVSSTSSLPLAALNMRVRRRLSLFLNVRTQVAADWTALAEEMDFEYLEIRQLETQADPTGRLLDAWQGRPGASVGRLLELLTKLGRDDVLLELGPSIEEDCQKYILKQQQEEAEKPLQVAAVDSSVPRTAELAGITTLDDPLGHMPERFDAFICYCPSDIQFVQEMIRQLEQTNYRLKLCVSDRDVLPGTCVWSIASELIEKRCRRMVVVVSDDYLQSKECDFQTKFALSLSPGAHQKRLIPIKYKAMKKEFPSILRFITVCDYTNPCTKSWFWTRLAKALSLP